European Patent Specification EP 3 606 542 B1, published June 10, 2026. Title: PROTEINS FOR THE TREATMENT OF EPITHELIAL BARRIER FUNCTION DISORDERS. Applicant: Second Genome, Inc. Han, Andrew Wonhee Goodyear, Andrew Whitman Gujral, Tarunmeet DeSantis, Todd Zachary Dabbagh, Karim Takeuchi, Toshihiko Jin, Ye Willcoxon, Michi Izumi Banas, Stefanie. The sequence listing filed with the application follows.

SEQUENCE LISTING (34 sequences)

SEQ ID NO: 1 - protein, 256 aa, Roseburia hominis
MKRLVCTVCSVLLCAGLLSGCGTSLEGEESVVYVGKKGVIASLDVETLDQSYYDETELKSYVDAEVEDYTAEHGKNAVKVESLKVEDGVAKLKMKYKTPEDYTAFNGIELYQGKVVASLAAGYVYDGEFARVEEGKVVGAATKQDIYSEDDLKVAIIRANTDVKVDGEICYVSCQNVKLTGKDSVSIRDGYYLETGSVTASVDVTGQESVGTEQLSGTEQMEMTGEPVNADDTEQTEAAAGDGSFETDVYTFIVYK

SEQ ID NO: 2 - DNA, 768 bp, Roseburia hominis
atgaagagattagtgtgcacggtctgcagtgtactgttgtgtgcgggacttctctccggatgcggtacctcgctggagggagaggaaagtgtcgtgtacgtgggaaagaaaggcgtgatagcgtcgctggatgtggagacgctcgatcagtcctactacgatgagacggaactgaagtcctatgtggatgcagaggtggaagattacaccgcggagcatggtaaaaatgcagtcaaggtggagagccttaaggtggaagacggtgtggcgaagcttaagatgaagtacaagacaccggaggattataccgcatttaatggaattgaactctatcaggggaaagtcgttgcttccctggcggcaggatacgtctacgacggggagttcgcccgcgtggaggaaggcaaggttgtgggagctgccacaaaacaggatatttactctgaggatgatttgaaagttgccatcatccgtgccaatacggatgtgaaggtggacggtgagatctgctatgtctcctgtcagaatgtgaagctgaccggaaaagacagtgtgtcgatccgtgacggatattatcttgagacgggaagcgtgacggcatccgtggatgtgaccggacaggagagcgtcgggaccgagcagctttcgggaaccgaacagatggagatgaccggggagccggtgaatgcggatgataccgagcagacagaggcggcggccggtgacggttcgttcgagacagacgtatatactttcattgtctacaaa

SEQ ID NO: 3 - protein, 232 aa, Roseburia hominis
LEGEESVVYVGKKGVIASLDVETLDQSYYDETELKSYVDAEVEDYTAEHGKNAVKVESLKVEDGVAKLKMKYKTPEDYTAFNGIELYQGKVVASLAAGYVYDGEFARVEEGKVVGAATKQDIYSEDDLKVAIIRANTDVKVDGEICYVSCQNVKLTGKDSVSIRDGYYLETGSVTASVDVTGQESVGTEQLSGTEQMEMTGEPVNADDTEQTEAAAGDGSFETDVYTFIVYK

SEQ ID NO: 4 - DNA, 696 bp, Roseburia hominis
ctggagggagaggaaagtgtcgtgtacgtgggaaagaaaggcgtgatagcgtcgctggatgtggagacgctcgatcagtcctactacgatgagacggaactgaagtcctatgtggatgcagaggtggaagattacaccgcggagcatggtaaaaatgcagtcaaggtggagagccttaaggtggaagacggtgtggcgaagcttaagatgaagtacaagacaccggaggattataccgcatttaatggaattgaactctatcaggggaaagtcgttgcttccctggcggcaggatacgtctacgacggggagttcgcccgcgtggaggaaggcaaggttgtgggagctgccacaaaacaggatatttactctgaggatgatttgaaagttgccatcatccgtgccaatacggatgtgaaggtggacggtgagatctgctatgtctcctgtcagaatgtgaagctgaccggaaaagacagtgtgtcgatccgtgacggatattatcttgagacgggaagcgtgacggcatccgtggatgtgaccggacaggagagcgtcgggaccgagcagctttcgggaaccgaacagatggagatgaccggggagccggtgaatgcggatgataccgagcagacagaggcggcggccggtgacggttcgttcgagacagacgtatatactttcattgtctacaaa

SEQ ID NO: 5 - protein, 241 aa, Artificial Sequence
  SG11 expressed in pGEX6 vector and cleaved by Precision protease
GPLGSLEGEESVVYVGKKGVIASLDVETLDQSYYDETELKSYVDAEVEDYTAEHGKNAVKVESLKVEDGVAKLKMKYKTPEDYTAFNGIELYQGKVVASLAAGYVYDGEFARVEEGKVVGAATKQDIYSEDDLKVAIIRANTDVKVDGEICYVSCQNVKLTGKDSVSIRDGYYLETGSVTASVDVTGQESVGTEQLSGTEQMEMTGEPVNADDTEQTEAAAGDGSFETDVYTFIVYKAAAS

SEQ ID NO: 6 - DNA, 723 bp, Artificial Sequence
  SG11 expressed in pGEX6 vector and cleaved by Precision protease
gggcccctgggatccctggagggagaggaaagtgtcgtgtacgtgggaaagaaaggcgtgatagcgtcgctggatgtggagacgctcgatcagtcctactacgatgagacggaactgaagtcctatgtggatgcagaggtggaagattacaccgcggagcatggtaaaaatgcagtcaaggtggagagccttaaggtggaagacggtgtggcgaagcttaagatgaagtacaagacaccggaggattataccgcatttaatggaattgaactctatcaggggaaagtcgttgcttccctggcggcaggatacgtctacgacggggagttcgcccgcgtggaggaaggcaaggttgtgggagctgccacaaaacaggatatttactctgaggatgatttgaaagttgccatcatccgtgccaatacggatgtgaaggtggacggtgagatctgctatgtctcctgtcagaatgtgaagctgaccggaaaagacagtgtgtcgatccgtgacggatattatcttgagacgggaagcgtgacggcatccgtggatgtgaccggacaggagagcgtcgggaccgagcagctttcgggaaccgaacagatggagatgaccggggagccggtgaatgcggatgataccgagcagacagaggcggcggccggtgacggttcgttcgagacagacgtatatactttcattgtctacaaagcggccgcatcg

SEQ ID NO: 7 - protein, 233 aa, Artificial Sequence
  SG11 with start methionine
MLEGEESVVYVGKKGVIASLDVETLDQSYYDETELKSYVDAEVEDYTAEHGKNAVKVESLKVEDGVAKLKMKYKTPEDYTAFNGIELYQGKVVASLAAGYVYDGEFARVEEGKVVGAATKQDIYSEDDLKVAIIRANTDVKVDGEICYVSCQNVKLTGKDSVSIRDGYYLETGSVTASVDVTGQESVGTEQLSGTEQMEMTGEPVNADDTEQTEAAAGDGSFETDVYTFIVYK

SEQ ID NO: 8 - DNA, 699 bp, Artificial Sequence
  SG11 with start methionine
atgttggagggtgaagagtctgttgtctatgtgggtaagaaaggtgtgatcgcgtccctggacgtcgagactctggaccagtcttactatgatgaaaccgagctgaagtcgtatgtggacgccgaagttgaggattacacggccgagcacggcaaaaatgccgtcaaagttgagagcttgaaagttgaggacggcgtggcaaagctgaagatgaaatacaagaccccagaggactacacggcgttcaatggtatcgagctgtatcagggcaaagtcgtcgcatccctggcagcgggctatgtgtacgacggtgagtttgcgcgcgtcgaagaaggcaaagttgtgggtgcggctacgaaacaagatatctacagcgaagatgacctgaaagtcgcgattattcgtgctaacaccgatgttaaagttgatggcgagatttgctacgttagctgtcaaaacgtaaagctgacgggtaaagatagcgtgagcattcgtgatggctattatctggaaaccggtagcgttacggcgagcgtcgatgttaccggtcaagagagcgtgggtaccgaacagctgagcggcaccgaacagatggaaatgaccggtgaaccggttaacgcagacgacacggaacaaaccgaagccgcggcaggcgacggtagcttcgagactgacgtgtacacctttatcgtgtacaag

SEQ ID NO: 9 - protein, 246 aa, Artificial Sequence
  SG11 with N-terminal FLAG tag
MDYKDDDDKGSSHMLEGEESVVYVGKKGVIASLDVETLDQSYYDETELKSYVDAEVEDYTAEHGKNAVKVESLKVEDGVAKLKMKYKTPEDYTAFNGIELYQGKVVASLAAGYVYDGEFARVEEGKVVGAATKQDIYSEDDLKVAIIRANTDVKVDGEICYVSCQNVKLTGKDSVSIRDGYYLETGSVTASVDVTGQESVGTEQLSGTEQMEMTGEPVNADDTEQTEAAAGDGSFETDVYTFIVYK

SEQ ID NO: 10 - DNA, 738 bp, Artificial Sequence
  SG11 with N-terminal FLAG tag (not codon optimized)
atggactacaaagacgatgacgacaagggcagcagccatatgctggagggagaggaaagtgtcgtgtacgtgggaaagaaaggcgtgatagcgtcgctggatgtggagacgctcgatcagtcctactacgatgagacggaactgaagtcctatgtggatgcagaggtggaagattacaccgcggagcatggtaaaaatgcagtcaaggtggagagccttaaggtggaagacggtgtggcgaagcttaagatgaagtacaagacaccggaggattataccgcatttaatggaattgaactctatcaggggaaagtcgttgcttccctggcggcaggatacgtctacgacggggagttcgcccgcgtggaggaaggcaaggttgtgggagctgccacaaaacaggatatttactctgaggatgatttgaaagttgccatcatccgtgccaatacggatgtgaaggtggacggtgagatctgctatgtctcctgtcagaatgtgaagctgaccggaaaagacagtgtgtcgatccgtgacggatattatcttgagacgggaagcgtgacggcatccgtggatgtgaccggacaggagagcgtcgggaccgagcagctttcgggaaccgaacagatggagatgaccggggagccggtgaatgcggatgataccgagcagacagaggcggcggccggtgacggttcgttcgagacagacgtatatactttcattgtctacaaa

SEQ ID NO: 11 - protein, 233 aa, Artificial Sequence
  Artificial variant of SG11  (C147V, C151S)
MLEGEESVVYVGKKGVIASLDVETLDQSYYDETELKSYVDAEVEDYTAEHGKNAVKVESLKVEDGVAKLKMKYKTPEDYTAFNGIELYQGKVVASLAAGYVYDGEFARVEEGKVVGAATKQDIYSEDDLKVAIIRANTDVKVDGEIVYVSSQNVKLTGKDSVSIRDGYYLETGSVTASVDVTGQESVGTEQLSGTEQMEMTGEPVNADDTEQTEAAAGDGSFETDVYTFIVYK

SEQ ID NO: 12 - DNA, 699 bp, Artificial Sequence
  Artificial variant of SG11  (C147V, C151S) (codon optimized)
atgttggagggtgaagagtctgttgtctatgtgggtaagaaaggtgtgatcgcgtccctggacgtcgagactctggaccagtcttactatgatgaaaccgagctgaagtcgtatgtggacgccgaagttgaggattacacggccgagcacggcaaaaatgccgtcaaagttgagagcttgaaagttgaggacggcgtggcaaagctgaagatgaaatacaagaccccagaggactacacggcgttcaatggtatcgagctgtatcagggcaaagtcgtcgcatccctggcagcgggctatgtgtacgacggtgagtttgcgcgcgtcgaagaaggcaaagttgtgggtgcggctacgaaacaagatatctacagcgaagatgacctgaaagtcgcgattattcgtgctaacaccgatgttaaagttgatggcgagattgtgtacgttagcagccaaaacgtaaagctgacgggtaaagatagcgtgagcattcgtgatggctattatctggaaaccggtagcgttacggcgagcgtcgatgttaccggtcaagagagcgtgggtaccgaacagctgagcggcaccgaacagatggaaatgaccggtgaaccggttaacgcagacgacacggaacaaaccgaagccgcggcaggcgacggtagcttcgagactgacgtgtacacctttatcgtgtacaag

SEQ ID NO: 13 - protein, 233 aa, Artificial Sequence
  Artificial variant of SG11  (G84D, C147V, C151S)
MLEGEESVVYVGKKGVIASLDVETLDQSYYDETELKSYVDAEVEDYTAEHGKNAVKVESLKVEDGVAKLKMKYKTPEDYTAFNDIELYQGKVVASLAAGYVYDGEFARVEEGKVVGAATKQDIYSEDDLKVAIIRANTDVKVDGEIVYVSSQNVKLTGKDSVSIRDGYYLETGSVTASVDVTGQESVGTEQLSGTEQMEMTGEPVNADDTEQTEAAAGDGSFETDVYTFIVYK

SEQ ID NO: 14 - DNA, 699 bp, Artificial Sequence
  Artificial variant of SG11  (G84D, C147V, C151S) (codon optimized)
atgttggagggtgaagagtctgttgtctatgtgggtaagaaaggtgtgatcgcgtccctggacgtcgagactctggaccagtcttactatgatgaaaccgagctgaagtcgtatgtggacgccgaagttgaggattacacggccgagcacggcaaaaatgccgtcaaagttgagagcttgaaagttgaggacggcgtggcaaagctgaagatgaaatacaagaccccagaggactacacggcgttcaatgacatcgagctgtatcagggcaaagtcgtcgcatccctggcagcgggctatgtgtacgacggtgagtttgcgcgcgtcgaagaaggcaaagttgtgggtgcggctacgaaacaagatatctacagcgaagatgacctgaaagtcgcgattattcgtgctaacaccgatgttaaagttgatggcgagattgtgtacgttagcagccaaaacgtaaagctgacgggtaaagatagcgtgagcattcgtgatggctattatctggaaaccggtagcgttacggcgagcgtcgatgttaccggtcaagagagcgtgggtaccgaacagctgagcggcaccgaacagatggaaatgaccggtgaaccggttaacgcagacgacacggaacaaaccgaagccgcggcaggcgacggtagcttcgagactgacgtgtacacctttatcgtgtacaag

SEQ ID NO: 15 - protein, 233 aa, Artificial Sequence
  Artificial variant of SG11  (N83S, C147V, C151S)
MLEGEESVVYVGKKGVIASLDVETLDQSYYDETELKSYVDAEVEDYTAEHGKNAVKVESLKVEDGVAKLKMKYKTPEDYTAFSGIELYQGKVVASLAAGYVYDGEFARVEEGKVVGAATKQDIYSEDDLKVAIIRANTDVKVDGEIVYVSSQNVKLTGKDSVSIRDGYYLETGSVTASVDVTGQESVGTEQLSGTEQMEMTGEPVNADDTEQTEAAAGDGSFETDVYTFIVYK

SEQ ID NO: 16 - DNA, 699 bp, Artificial Sequence
  Artificial variant of SG11  (N83S, C147V, C151S) (codon optimized)
atgttggagggtgaagagtctgttgtctatgtgggtaagaaaggtgtgatcgcgtccctggacgtcgagactctggaccagtcttactatgatgaaaccgagctgaagtcgtatgtggacgccgaagttgaggattacacggccgagcacggcaaaaatgccgtcaaagttgagagcttgaaagttgaggacggcgtggcaaagctgaagatgaaatacaagaccccagaggactacacggcgttcagcggtatcgagctgtatcagggcaaagtcgtcgcatccctggcagcgggctatgtgtacgacggtgagtttgcgcgcgtcgaagaaggcaaagttgtgggtgcggctacgaaacaagatatctacagcgaagatgacctgaaagtcgcgattattcgtgctaacaccgatgttaaagttgatggcgagattgtgtacgttagcagccaaaacgtaaagctgacgggtaaagatagcgtgagcattcgtgatggctattatctggaaaccggtagcgttacggcgagcgtcgatgttaccggtcaagagagcgtgggtaccgaacagctgagcggcaccgaacagatggaaatgaccggtgaaccggttaacgcagacgacacggaacaaaccgaagccgcggcaggcgacggtagcttcgagactgacgtgtacacctttatcgtgtacaag

SEQ ID NO: 17 - protein, 233 aa, Artificial Sequence
  Artificial variant of SG11  (N53S, G84D, C147V, C151S)
MLEGEESVVYVGKKGVIASLDVETLDQSYYDETELKSYVDAEVEDYTAEHGKSAVKVESLKVEDGVAKLKMKYKTPEDYTAFNDIELYQGKVVASLAAGYVYDGEFARVEEGKVVGAATKQDIYSEDDLKVAIIRANTDVKVDGEIVYVSSQNVKLTGKDSVSIRDGYYLETGSVTASVDVTGQESVGTEQLSGTEQMEMTGEPVNADDTEQTEAAAGDGSFETDVYTFIVYK

SEQ ID NO: 18 - DNA, 699 bp, Artificial Sequence
  Artificial variant of SG11  (N53S, G84D, C147V, C151S) (codon optimized)
atgttggagggtgaagagtctgttgtctatgtgggtaagaaaggtgtgatcgcgtccctggacgtcgagactctggaccagtcttactatgatgaaaccgagctgaagtcgtatgtggacgccgaagttgaggattacacggccgagcacggcaaatccgccgtcaaagttgagagcttgaaagttgaggacggcgtggcaaagctgaagatgaaatacaagaccccagaggactacacggcgttcaatgacatcgagctgtatcagggcaaagtcgtcgcatccctggcagcgggctatgtgtacgacggtgagtttgcgcgcgtcgaagaaggcaaagttgtgggtgcggctacgaaacaagatatctacagcgaagatgacctgaaagtcgcgattattcgtgctaacaccgatgttaaagttgatggcgagattgtgtacgttagcagccaaaacgtaaagctgacgggtaaagatagcgtgagcattcgtgatggctattatctggaaaccggtagcgttacggcgagcgtcgatgttaccggtcaagagagcgtgggtaccgaacagctgagcggcaccgaacagatggaaatgaccggtgaaccggttaacgcagacgacacggaacaaaccgaagccgcggcaggcgacggtagcttcgagactgacgtgtacacctttatcgtgtacaag

SEQ ID NO: 19 - protein, 233 aa, Artificial Sequence
  Artificial variant of SG11  (N53S, N83S, C147V, C151S)
MLEGEESVVYVGKKGVIASLDVETLDQSYYDETELKSYVDAEVEDYTAEHGKSAVKVESLKVEDGVAKLKMKYKTPEDYTAFSGIELYQGKVVASLAAGYVYDGEFARVEEGKVVGAATKQDIYSEDDLKVAIIRANTDVKVDGEIVYVSSQNVKLTGKDSVSIRDGYYLETGSVTASVDVTGQESVGTEQLSGTEQMEMTGEPVNADDTEQTEAAAGDGSFETDVYTFIVYK

SEQ ID NO: 20 - DNA, 699 bp, Artificial Sequence
  Artificial variant of SG11  (N53S, N83S, C147V, C151S) (codon optimized)
atgttggagggtgaagagtctgttgtctatgtgggtaagaaaggtgtgatcgcgtccctggacgtcgagactctggaccagtcttactatgatgaaaccgagctgaagtcgtatgtggacgccgaagttgaggattacacggccgagcacggcaaatccgccgtcaaagttgagagcttgaaagttgaggacggcgtggcaaagctgaagatgaaatacaagaccccagaggactacacggcgttcagcggtatcgagctgtatcagggcaaagtcgtcgcatccctggcagcgggctatgtgtacgacggtgagtttgcgcgcgtcgaagaaggcaaagttgtgggtgcggctacgaaacaagatatctacagcgaagatgacctgaaagtcgcgattattcgtgctaacaccgatgttaaagttgatggcgagattgtgtacgttagcagccaaaacgtaaagctgacgggtaaagatagcgtgagcattcgtgatggctattatctggaaaccggtagcgttacggcgagcgtcgatgttaccggtcaagagagcgtgggtaccgaacagctgagcggcaccgaacagatggaaatgaccggtgaaccggttaacgcagacgacacggaacaaaccgaagccgcggcaggcgacggtagcttcgagactgacgtgtacacctttatcgtgtacaag

SEQ ID NO: 21 - protein, 227 aa, Roseburia intestinalis
MLDADTDTVYVQKNGTVLSVDVETLDKDYYDETELKDYVTDAVSTYTGEHGKSAVKLENLSVKDGTATLKMKYKTPEDYTGFNGIELYEGKVVKALAAGYDFKTDFVSVEDGKVTGTATKEEIYSGEDLKVVIIKANRDVKVDGTICYVSSENVKLTGTDSVSIRDGYSLNSGSTADESDSDENIADGTESIGGSTEVSDTDVNDDTTYVKDDGAFETDVYTYIIYK

SEQ ID NO: 22 - protein, 215 aa, Roseburia sp. 831b
MLDVEESTVYVQKNGSVISTDIEDFSADYYDEDELKDYIGDEISSYTSENGKKSVSLESVSVKDSVAKLTMKYKTAEDYTNFNGVELYTGTIVKAMAAGYDFGVDFVSVKDGAVTGTATKDEIVDHDDYKVAVIKANTDVKVDGTIVYVSSQNVKVTGKNTVSIREGYLAADTTNVVGSTETVAETEAEEANQTEAVLEDEFASESDVYTYVIFK

SEQ ID NO: 23 - protein, 236 aa, Roseburia inulinivorans
MLEADTNTVYVSKHGKVVSMDVEQLDQSYYDETELKEFVDSAVDEYNTENGKNSVKVDDLTVEDGTAKLRMDYETVDDYTAFNGVELYEGKIVQALAAGYDFDTDFAGVDKDGCVTGVTRGDILAQEDLKVVIIKANTDVKIDGKILYVSCDNVTVTGKDSVSIKEGTGIEKTWITEAEEVPSTEAVLETESTEDAGDVIEGEVIIGTEEASGNDVVTNLSGGSSGTDVYTYIIYK

SEQ ID NO: 24 - protein, 13 aa, Artificial Sequence
  Fragment of SG11 with start methionine
MLEGEESVVYVGK

SEQ ID NO: 25 - protein, 22 aa, Roseburia hominis
GVIASLDVETLDQSYYDETELK

SEQ ID NO: 26 - protein, 17 aa, Roseburia hominis
TPEDYTAFNGIELYQGK

SEQ ID NO: 27 - protein, 6 aa, Roseburia hominis
ANTDVK

SEQ ID NO: 28 - protein, 14 aa, Roseburia hominis
VDGEICYVSCQNVK

SEQ ID NO: 29 - protein, 67 aa, Roseburia hominis
GYYLETGSVTASVDVTGQESVGTEQLSGTEQMEMTGEPVNADDTEQTEAAAGDGSFETDVYTFIVYK

SEQ ID NO: 30 - protein, 4 aa, Roseburia hominis
NAVK

SEQ ID NO: 31 - protein, 17 aa, Roseburia hominis
TPEDYTAFSGIELYQGK

SEQ ID NO: 32 - protein, 8 aa, Artificial Sequence
  FLAG tag
DYKDDDDK

SEQ ID NO: 33 - protein, 233 aa, Artificial Sequence
  Artificial variant of SG11
  misc_feature (53)..(53): Xaa can be any naturally occurring amino acid
  misc_feature (83)..(84): Xaa can be any naturally occurring amino acid
  misc_feature (147)..(147): Xaa can be any naturally occurring amino acid
  misc_feature (151)..(151): Xaa can be any naturally occurring amino acid
MLEGEESVVYVGKKGVIASLDVETLDQSYYDETELKSYVDAEVEDYTAEHGKXAVKVESLKVEDGVAKLKMKYKTPEDYTAFXXIELYQGKVVASLAAGYVYDGEFARVEEGKVVGAATKQDIYSEDDLKVAIIRANTDVKVDGEIXYVSXQNVKLTGKDSVSIRDGYYLETGSVTASVDVTGQESVGTEQLSGTEQMEMTGEPVNADDTEQTEAAAGDGSFETDVYTFIVYK

SEQ ID NO: 34 - protein, 233 aa, Artificial Sequence; identical to SEQ ID NO: 33
  Artificial variant of SG11
  misc_feature (53)..(53): Xaa is any amino acid other than Asn
  misc_feature (83)..(83): Xaa is any amino acid other than Asn
  misc_feature (84)..(84): Xaa is any amino acid other than Gly
  misc_feature (147)..(147): Xaa is any amino acid other than Cys
  misc_feature (151)..(151): Xaa is any amino acid other than Cys